European Patent Application EP 4 509 603 A1, published February 19, 2025. Title: NEW APTAMERS AGAINST EphA2 (ephrin type-A receptor 2). Applicant: Aptadel Therapeutics SL. The sequence listing filed with the application follows.

SEQUENCE LISTING (148 sequences)

SEQ ID NO: 1 - RNA, 49 nt, synthetic construct
  source 1..49: mol_type = other RNA; note = Apt1 sequence
  modified_base 1..49: mod_base = OTHER; note = All pyrimidines are 2-fluoro-modified pyrimidines
gggaggacgatgcggtcctgcgtctgttcgtccccagacgctcgcccga

SEQ ID NO: 2 - RNA, 47 nt, synthetic construct
  source 1..47: mol_type = other RNA; note = Apt2 sequence
  modified_base 1..47: mod_base = OTHER; note = All pyrimidines are 2-fluoro-modified pyrimidines
gggaggacgatgcggtcctgcgctgttcgtccccagcgctcgcccga

SEQ ID NO: 3 - RNA, 47 nt, synthetic construct
  source 1..47: mol_type = other RNA; note = Apt3 sequence
  modified_base 1..47: mod_base = OTHER; note = All pyrimidines are 2-fluoro-modified pyrimidines
gggaggacgatgcggtcctgcgtcgttcgtccccgacgctcgcccga

SEQ ID NO: 4 - RNA, 47 nt, synthetic construct
  source 1..47: mol_type = other RNA; note = Apt4 sequence
  modified_base 1..47: mod_base = OTHER; note = All pyrimidines are 2-fluoro-modified pyrimidines
gggaggacgatgcggtcctgtcctgttcgtccccaggactcgcccga

SEQ ID NO: 5 - RNA, 45 nt, synthetic construct
  source 1..45: mol_type = other RNA; note = Apt5 sequence
  modified_base 1..45: mod_base = OTHER; note = All pyrimidines are 2-fluoro-modified pyrimidines
gggaggacgatgcggtcctgcgcgttcgtccccgcgctcgcccga

SEQ ID NO: 6 - RNA, 45 nt, synthetic construct
  source 1..45: mol_type = other RNA; note = Apt6 sequence
  modified_base 1..45: mod_base = OTHER; note = All pyrimidines are 2-fluoro-modified pyrimidines
gggaggacgatgcggtcctgtctgttcgtccccagactcgcccga

SEQ ID NO: 7 - RNA, 49 nt, synthetic construct
  source 1..49: mol_type = other RNA; note = Apt7 sequence
  modified_base 1..49: mod_base = OTHER; note = All pyrimidines are 2-fluoro-modified pyrimidines
gggaggacgatgcggtcctgtcgtctgttcgtccccagacgactcgccc

SEQ ID NO: 8 - RNA, 43 nt, synthetic construct
  source 1..43: mol_type = other RNA; note = Apt8 sequence
  modified_base 1..43: mod_base = OTHER; note = All pyrimidines are 2-fluoro-modified pyrimidines
aggacgatgcggtcctgtcgtctgttcgtccccagacgactcg

SEQ ID NO: 9 - RNA, 42 nt, synthetic construct
  source 1..42: mol_type = other RNA; note = Apt9 sequence
  modified_base 1..42: mod_base = OTHER; note = All pyrimidines are 2-fluoro-modified pyrimidines
ggacgatgcggtcctgtcgtctgttcgtccccagacgactcg

SEQ ID NO: 10 - RNA, 44 nt, synthetic construct
  source 1..44: mol_type = other RNA; note = Apt10 sequence
  modified_base 1..44: mod_base = OTHER; note = All pyrimidines are 2-fluoro-modified pyrimidines
cggacgatgcggtccgtgtcgtctgttcgtccccagacgactcg

SEQ ID NO: 11 - RNA, 50 nt, synthetic construct
  source 1..50: mol_type = other RNA; note = Apt11 sequence
  modified_base 1..50: mod_base = OTHER; note = All pyrimidines are 2-fluoro-modified pyrimidines
gggaggacatgcggtcctgtcgtctgttcgtccccagacgactcgcccga

SEQ ID NO: 12 - RNA, 50 nt, synthetic construct
  source 1..50: mol_type = other RNA; note = Apt12 sequence
  modified_base 1..50: mod_base = OTHER; note = All pyrimidines are 2-fluoro-modified pyrimidines
gggaggacgtgcggtcctgtcgtctgttcgtccccagacgactcgcccga

SEQ ID NO: 13 - RNA, 50 nt, synthetic construct
  source 1..50: mol_type = other RNA; note = Apt13 sequence
  modified_base 1..50: mod_base = OTHER; note = All pyrimidines are 2-fluoro-modified pyrimidines
gggaggacgagcggtcctgtcgtctgttcgtccccagacgactcgcccga

SEQ ID NO: 14 - RNA, 50 nt, synthetic construct
  source 1..50: mol_type = other RNA; note = Apt14 sequence
  modified_base 1..50: mod_base = OTHER; note = All pyrimidines are 2-fluoro-modified pyrimidines
gggaggacgatcggtcctgtcgtctgttcgtccccagacgactcgcccga

SEQ ID NO: 15 - RNA, 50 nt, synthetic construct
  source 1..50: mol_type = other RNA; note = Apt15 sequence
  modified_base 1..50: mod_base = OTHER; note = All pyrimidines are 2-fluoro-modified pyrimidines
gggaggacgatgggtcctgtcgtctgttcgtccccagacgactcgcccga

SEQ ID NO: 16 - RNA, 49 nt, synthetic construct
  source 1..49: mol_type = other RNA; note = Apt16 sequence
  modified_base 1..49: mod_base = OTHER; note = All pyrimidines are 2-fluoro-modified pyrimidines
gggaggacgatgcggtcctgtcgctgttcgtccccagcgactcgcccga

SEQ ID NO: 17 - RNA, 50 nt, synthetic construct
  source 1..50: mol_type = other RNA; note = Apt17 sequence
  modified_base 1..50: mod_base = OTHER; note = All pyrimidines are 2-fluoro-modified pyrimidines
gggaggacgatgcgtcctgtcgtctgttcgtccccagacgactcgcccga

SEQ ID NO: 18 - RNA, 50 nt, synthetic construct
  source 1..50: mol_type = other RNA; note = Apt18 sequence
  modified_base 1..50: mod_base = OTHER; note = All pyrimidines are 2-fluoro-modified pyrimidines
gggaggacgatgcggtcctgtcgtctgtcgtccccagacgactcgcccga

SEQ ID NO: 19 - RNA, 50 nt, synthetic construct
  source 1..50: mol_type = other RNA; note = Apt19 sequence
  modified_base 1..50: mod_base = OTHER; note = All pyrimidines are 2-fluoro-modified pyrimidines
gggaggacgatgcggtcctgtcgtctgttgtccccagacgactcgcccga

SEQ ID NO: 20 - RNA, 50 nt, synthetic construct
  source 1..50: mol_type = other RNA; note = Apt20 sequence
  modified_base 1..50: mod_base = OTHER; note = All pyrimidines are 2-fluoro-modified pyrimidines
gggaggacgatgcggtcctgtcgtctgttctccccagacgactcgcccga

SEQ ID NO: 21 - RNA, 50 nt, synthetic construct
  source 1..50: mol_type = other RNA; note = Apt21 sequence
  modified_base 1..50: mod_base = OTHER; note = All pyrimidines are 2-fluoro-modified pyrimidines
gggaggacgatgcggtcctgtcgtctgttcgccccagacgactcgcccga

SEQ ID NO: 22 - RNA, 42 nt, synthetic construct
  source 1..42: mol_type = other RNA; note = Apt22 sequence
  modified_base 1..42: mod_base = OTHER; note = All pyrimidines are 2-fluoro-modified pyrimidines
cggacgatgcggtccgtgcgtctgttcgtccccagacgctcg

SEQ ID NO: 23 - RNA, 42 nt, synthetic construct
  source 1..42: mol_type = other RNA; note = Apt23 sequence
  modified_base 1..42: mod_base = OTHER; note = All pyrimidines are 2-fluoro-modified pyrimidines
cggacgatgcggtccgtgtcgctgttcgtccccagcgactcg

SEQ ID NO: 24 - RNA, 42 nt, synthetic construct
  source 1..42: mol_type = other RNA; note = Apt24 sequence
  modified_base 1..42: mod_base = OTHER; note = All pyrimidines are 2-fluoro-modified pyrimidines
cggacgatgcggtccgtgtcgtcgttcgtccccgacgactcg

SEQ ID NO: 25 - RNA, 40 nt, synthetic construct
  source 1..40: mol_type = other RNA; note = Apt25 sequence
  modified_base 1..40: mod_base = OTHER; note = All pyrimidines are 2-fluoro-modified pyrimidines
cggacgatgcggtccgtgcgctgttcgtccccagcgctcg

SEQ ID NO: 26 - RNA, 40 nt, synthetic construct
  source 1..40: mol_type = other RNA; note = Apt26 sequence
  modified_base 1..40: mod_base = OTHER; note = All pyrimidines are 2-fluoro-modified pyrimidines
cggacgatgcggtccgtgcgtcgttcgtccccgacgctcg

SEQ ID NO: 27 - RNA, 40 nt, synthetic construct
  source 1..40: mol_type = other RNA; note = Apt27 sequence
  modified_base 1..40: mod_base = OTHER; note = All pyrimidines are 2-fluoro-modified pyrimidines
cggacgatgcggtccgtgtcgcgttcgtccccgcgactcg

SEQ ID NO: 28 - RNA, 38 nt, synthetic construct
  source 1..38: mol_type = other RNA; note = Apt28 sequence
  modified_base 1..38: mod_base = OTHER; note = All pyrimidines are 2-fluoro-modified pyrimidines
cggacgatgcggtccgtgcgcgttcgtccccgcgctcg

SEQ ID NO: 29 - RNA, 37 nt, synthetic construct
  source 1..37: mol_type = other RNA; note = Apt29 sequence
  modified_base 1..37: mod_base = OTHER; note = All pyrimidines are 2-fluoro-modified pyrimidines
cggacgatgcggtccgtgtcgcgttcgtccccgcgac

SEQ ID NO: 30 - RNA, 49 nt, synthetic construct
  source 1..49: mol_type = other RNA; note = Apt30 sequence
  modified_base 1..49: mod_base = OTHER; note = All pyrimidines are 2-fluoro-modified pyrimidines
gggaggacgacggtcctgtcgtctgttcgtccccagacgactcgcccga

SEQ ID NO: 31 - RNA, 49 nt, synthetic construct
  source 1..49: mol_type = other RNA; note = Apt31 sequence
  modified_base 1..49: mod_base = OTHER; note = All pyrimidines are 2-fluoro-modified pyrimidines
gggaggacgtcggtcctgtcgtctgttcgtccccagacgactcgcccga

SEQ ID NO: 32 - RNA, 49 nt, synthetic construct
  source 1..49: mol_type = other RNA; note = Apt32 sequence
  modified_base 1..49: mod_base = OTHER; note = All pyrimidines are 2-fluoro-modified pyrimidines
gggaggacatcggtcctgtcgtctgttcgtccccagacgactcgcccga

SEQ ID NO: 33 - RNA, 49 nt, synthetic construct
  source 1..49: mol_type = other RNA; note = Apt33 sequence
  modified_base 1..49: mod_base = OTHER; note = All pyrimidines are 2-fluoro-modified pyrimidines
gggaggacgatggtcctgtcgtctgttcgtccccagacgactcgcccga

SEQ ID NO: 34 - RNA, 48 nt, synthetic construct
  source 1..48: mol_type = other RNA; note = Apt34 sequence
  modified_base 1..48: mod_base = OTHER; note = All pyrimidines are 2-fluoro-modified pyrimidines
gggaggacgcggtcctgtcgtctgttcgtccccagacgactcgcccga

SEQ ID NO: 35 - RNA, 48 nt, synthetic construct
  source 1..48: mol_type = other RNA; note = Apt35 sequence
  modified_base 1..48: mod_base = OTHER; note = All pyrimidines are 2-fluoro-modified pyrimidines
gggaggacacggtcctgtcgtctgttcgtccccagacgactcgcccga

SEQ ID NO: 36 - RNA, 48 nt, synthetic construct
  source 1..48: mol_type = other RNA; note = Apt36 sequence
  modified_base 1..48: mod_base = OTHER; note = All pyrimidines are 2-fluoro-modified pyrimidines
gggaggacgaggtcctgtcgtctgttcgtccccagacgactcgcccga

SEQ ID NO: 37 - RNA, 47 nt, synthetic construct
  source 1..47: mol_type = other RNA; note = Apt37 sequence
  modified_base 1..47: mod_base = OTHER; note = All pyrimidines are 2-fluoro-modified pyrimidines
gggaggacgggtcctgtcgtctgttcgtccccagacgactcgcccga

SEQ ID NO: 38 - RNA, 47 nt, synthetic construct
  source 1..47: mol_type = other RNA; note = Apt38 sequence
  modified_base 1..47: mod_base = OTHER; note = All pyrimidines are 2-fluoro-modified pyrimidines
gggaggacaggtcctgtcgtctgttcgtccccagacgactcgcccga

SEQ ID NO: 39 - RNA, 46 nt, synthetic construct
  source 1..46: mol_type = other RNA; note = Apt39 sequence
  modified_base 1..46: mod_base = OTHER; note = All pyrimidines are 2-fluoro-modified pyrimidines
gggaggacggtcctgtcgtctgttcgtccccagacgactcgcccga

SEQ ID NO: 40 - RNA, 47 nt, synthetic construct
  source 1..47: mol_type = other RNA; note = Apt40 sequence
  modified_base 1..47: mod_base = OTHER; note = All pyrimidines are 2-fluoro-modified pyrimidines
gggaggacgatgcggtcctgctctgttcgtccccagagctcgcccga

SEQ ID NO: 41 - RNA, 47 nt, synthetic construct
  source 1..47: mol_type = other RNA; note = Apt41 sequence
  modified_base 1..47: mod_base = OTHER; note = All pyrimidines are 2-fluoro-modified pyrimidines
gggaggacgatgcggtcctgttctgttcgtccccagaactcgcccga

SEQ ID NO: 42 - RNA, 45 nt, synthetic construct
  source 1..45: mol_type = other RNA; note = Apt42 sequence
  modified_base 1..45: mod_base = OTHER; note = All pyrimidines are 2-fluoro-modified pyrimidines
gggaggacgatgcggtcctgcctgttcgtccccaggctcgcccga

SEQ ID NO: 43 - RNA, 45 nt, synthetic construct
  source 1..45: mol_type = other RNA; note = Apt43 sequence
  modified_base 1..45: mod_base = OTHER; note = All pyrimidines are 2-fluoro-modified pyrimidines
gggaggacgacggtcctgtcctgttcgtccccaggactcgcccga

SEQ ID NO: 44 - RNA, 46 nt, synthetic construct
  source 1..46: mol_type = other RNA; note = Apt44 sequence
  modified_base 1..46: mod_base = OTHER; note = All pyrimidines are 2-fluoro-modified pyrimidines
gggaggacgatcggtcctgctctgttcgtccccagagctcgcccga

SEQ ID NO: 45 - RNA, 45 nt, synthetic construct
  source 1..45: mol_type = other RNA; note = Apt45 sequence
  modified_base 1..45: mod_base = OTHER; note = All pyrimidines are 2-fluoro-modified pyrimidines
gggaggacgacggtcctgctctgttcgtccccagagctcgcccga

SEQ ID NO: 46 - RNA, 46 nt, synthetic construct
  source 1..46: mol_type = other RNA; note = Apt46 sequence
  modified_base 1..46: mod_base = OTHER; note = All pyrimidines are 2-fluoro-modified pyrimidines
gggaggacgatcggtcctgttctgttcgtccccagaactcgcccga

SEQ ID NO: 47 - RNA, 45 nt, synthetic construct
  source 1..45: mol_type = other RNA; note = Apt47 sequence
  modified_base 1..45: mod_base = OTHER; note = All pyrimidines are 2-fluoro-modified pyrimidines
gggaggacgacggtcctgttctgttcgtccccagaactcgcccga

SEQ ID NO: 48 - RNA, 43 nt, synthetic construct
  source 1..43: mol_type = other RNA; note = Apt48 sequence
  modified_base 1..43: mod_base = OTHER; note = All pyrimidines are 2-fluoro-modified pyrimidines
gggaggacgacggtcctgcctgttcgtccccaggctcgcccga

SEQ ID NO: 49 - RNA, 44 nt, synthetic construct
  source 1..44: mol_type = other RNA; note = Apt49 sequence
  modified_base 1..44: mod_base = OTHER; note = All pyrimidines are 2-fluoro-modified pyrimidines
gggaggacgatcggtcctgtctgttcgtccccagactcgcccga

SEQ ID NO: 50 - RNA, 43 nt, synthetic construct
  source 1..43: mol_type = other RNA; note = Apt50 sequence
  modified_base 1..43: mod_base = OTHER; note = All pyrimidines are 2-fluoro-modified pyrimidines
gggaggacgacggtcctgtctgttcgtccccagactcgcccga

SEQ ID NO: 51 - RNA, 44 nt, synthetic construct
  source 1..44: mol_type = other RNA; note = Apt51 sequence
  modified_base 1..44: mod_base = OTHER; note = All pyrimidines are 2-fluoro-modified pyrimidines
gggaggacgcggtcctgtcctgttcgtccccaggactcgcccga

SEQ ID NO: 52 - RNA, 43 nt, synthetic construct
  source 1..43: mol_type = other RNA; note = Apt52 sequence
  modified_base 1..43: mod_base = OTHER; note = All pyrimidines are 2-fluoro-modified pyrimidines
gggaggaccggtcctgtcctgttcgtccccaggactcgcccga

SEQ ID NO: 53 - RNA, 42 nt, synthetic construct
  source 1..42: mol_type = other RNA; note = Apt53 sequence
  modified_base 1..42: mod_base = OTHER; note = All pyrimidines are 2-fluoro-modified pyrimidines
gggaggacggtcctgtcctgttcgtccccaggactcgcccga

SEQ ID NO: 54 - RNA, 44 nt, synthetic construct
  source 1..44: mol_type = other RNA; note = Apt54 sequence
  modified_base 1..44: mod_base = OTHER; note = All pyrimidines are 2-fluoro-modified pyrimidines
ggaggacgatcggtcctgtcctgttcgtccccaggactcgccga

SEQ ID NO: 55 - RNA, 42 nt, synthetic construct
  source 1..42: mol_type = other RNA; note = Apt55 sequence
  modified_base 1..42: mod_base = OTHER; note = All pyrimidines are 2-fluoro-modified pyrimidines
gaggacgatcggtcctgtcctgttcgtccccaggactcgcga

SEQ ID NO: 56 - RNA, 35 nt, synthetic construct
  source 1..35: mol_type = other RNA; note = Apt56 sequence
  modified_base 1..35: mod_base = OTHER; note = All pyrimidines are 2-fluoro-modified pyrimidines
gggtcctgtcctgttcgtccccaggactcgcccga

SEQ ID NO: 57 - RNA, 32 nt, synthetic construct
  source 1..32: mol_type = other RNA; note = Apt57 sequence
  modified_base 1..32: mod_base = OTHER; note = All pyrimidines are 2-fluoro-modified pyrimidines
gggtgtcctgttcgtccccaggactcgcccga

SEQ ID NO: 58 - RNA, 31 nt, synthetic construct
  source 1..31: mol_type = other RNA; note = Apt58 sequence
  modified_base 1..31: mod_base = OTHER; note = All pyrimidines are 2-fluoro-modified pyrimidines
ggggtcctgttcgtccccaggactcgcccga

SEQ ID NO: 59 - RNA, 44 nt, synthetic construct
  source 1..44: mol_type = other RNA; note = Apt59 sequence
  modified_base 1..44: mod_base = OTHER; note = All pyrimidines are 2-fluoro-modified pyrimidines
gggaggcgatcggcctgtcctgttcgtccccaggactcgcccga

SEQ ID NO: 60 - RNA, 44 nt, synthetic construct
  source 1..44: mol_type = other RNA; note = Apt60 sequence
  modified_base 1..44: mod_base = OTHER; note = All pyrimidines are 2-fluoro-modified pyrimidines
gggagacgatcggtctgtcctgttcgtccccaggactcgcccga

SEQ ID NO: 61 - RNA, 42 nt, synthetic construct
  source 1..42: mol_type = other RNA; note = Apt61 sequence
  modified_base 1..42: mod_base = OTHER; note = All pyrimidines are 2-fluoro-modified pyrimidines
gggagcgatcggctgtcctgttcgtccccaggactcgcccga

SEQ ID NO: 62 - RNA, 47 nt, synthetic construct
  source 1..47: mol_type = other RNA; note = Apt62 sequence
  modified_base 1..47: mod_base = OTHER; note = All pyrimidines are 2-fluoro-modified pyrimidines
gggaggaccggtcctgtcgtctgttcgtccccagacgactcgcccga

SEQ ID NO: 63 - RNA, 46 nt, synthetic construct
  source 1..46: mol_type = other RNA; note = Apt63 sequence
  modified_base 1..46: mod_base = OTHER; note = All pyrimidines are 2-fluoro-modified pyrimidines
gggaggacgatcggtcctgtcctgttcgtccccaggactcgcccga

SEQ ID NO: 64 - RNA, 44 nt, synthetic construct
  source 1..44: mol_type = other RNA; note = Apt64 sequence
  modified_base 1..44: mod_base = OTHER; note = All pyrimidines are 2-fluoro-modified pyrimidines
gggaggacgatcggtcctgcctgttcgtccccaggctcgcccga

SEQ ID NO: 65 - RNA, 42 nt, synthetic construct
  source 1..42: mol_type = other RNA; note = Apt65 sequence
  modified_base 1..42: mod_base = OTHER; note = All pyrimidines are 2-fluoro-modified pyrimidines
gggaggacggtcctgttctgttcgtccccagaactcgcccga

SEQ ID NO: 66 - RNA, 40 nt, synthetic construct
  source 1..40: mol_type = other RNA; note = Apt66 sequence
  modified_base 1..40: mod_base = OTHER; note = All pyrimidines are 2-fluoro-modified pyrimidines
gggaggacggtcctgtctgttcgtccccagactcgcccga

SEQ ID NO: 67 - RNA, 42 nt, synthetic construct
  source 1..42: mol_type = other RNA; note = Apt67 sequence
  modified_base 1..42: mod_base = OTHER; note = All pyrimidines are 2-fluoro-modified pyrimidines
gaggacggtcctgtcgtctgttcgtccccagacgactcgcga

SEQ ID NO: 68 - RNA, 42 nt, synthetic construct
  source 1..42: mol_type = other RNA; note = Apt68 sequence
  modified_base 1..42: mod_base = OTHER; note = All pyrimidines are 2-fluoro-modified pyrimidines
gggagcggctgtcgtctgttcgtccccagacgactcgcccga

SEQ ID NO: 69 - RNA, 41 nt, synthetic construct
  source 1..41: mol_type = other RNA; note = Apt69 sequence
  modified_base 1..41: mod_base = OTHER; note = All pyrimidines are 2-fluoro-modified pyrimidines
ggagcgatgcggctgttctgttcgtccccagaactcgccga

SEQ ID NO: 70 - RNA, 39 nt, synthetic construct
  source 1..39: mol_type = other RNA; note = Apt70 sequence
  modified_base 1..39: mod_base = OTHER; note = All pyrimidines are 2-fluoro-modified pyrimidines
gagcgatgcggctgttctgttcgtccccagaactcgcga

SEQ ID NO: 71 - RNA, 41 nt, synthetic construct
  source 1..41: mol_type = other RNA; note = Apt71 sequence
  modified_base 1..41: mod_base = OTHER; note = All pyrimidines are 2-fluoro-modified pyrimidines
gaggacgatgcggtcctgtctgttcgtccccagactcgcga

SEQ ID NO: 72 - RNA, 41 nt, synthetic construct
  source 1..41: mol_type = other RNA; note = Apt72 sequence
  modified_base 1..41: mod_base = OTHER; note = All pyrimidines are 2-fluoro-modified pyrimidines
gggagcgatgcggctgtctgttcgtccccagactcgcccga

SEQ ID NO: 73 - RNA, 39 nt, synthetic construct
  source 1..39: mol_type = other RNA; note = Apt73 sequence
  modified_base 1..39: mod_base = OTHER; note = All pyrimidines are 2-fluoro-modified pyrimidines
ggagcgatgcggctgtctgttcgtccccagactcgccga

SEQ ID NO: 74 - RNA, 37 nt, synthetic construct
  source 1..37: mol_type = other RNA; note = Apt74 sequence
  modified_base 1..37: mod_base = OTHER; note = All pyrimidines are 2-fluoro-modified pyrimidines
gagcgatgcggctgtctgttcgtccccagactcgcga

SEQ ID NO: 75 - RNA, 42 nt, synthetic construct
  source 1..42: mol_type = other RNA; note = Apt75 sequence
  modified_base 1..42: mod_base = OTHER; note = All pyrimidines are 2-fluoro-modified pyrimidines
ggaggacgatcggtcctgtctgttcgtccccagactcgccga

SEQ ID NO: 76 - RNA, 42 nt, synthetic construct
  source 1..42: mol_type = other RNA; note = Apt76 sequence
  modified_base 1..42: mod_base = OTHER; note = All pyrimidines are 2-fluoro-modified pyrimidines
gaggacgatcggtcctgttctgttcgtccccagaactcgcga

SEQ ID NO: 77 - RNA, 40 nt, synthetic construct
  source 1..40: mol_type = other RNA; note = Apt77 sequence
  modified_base 1..40: mod_base = OTHER; note = All pyrimidines are 2-fluoro-modified pyrimidines
gaggacgatcggtcctgtctgttcgtccccagactcgcga

SEQ ID NO: 78 - RNA, 42 nt, synthetic construct
  source 1..42: mol_type = other RNA; note = Apt78 sequence
  modified_base 1..42: mod_base = OTHER; note = All pyrimidines are 2-fluoro-modified pyrimidines
gggagcgatcggctgttctgttcgtccccagaactcgcccga

SEQ ID NO: 79 - RNA, 40 nt, synthetic construct
  source 1..40: mol_type = other RNA; note = Apt79 sequence
  modified_base 1..40: mod_base = OTHER; note = All pyrimidines are 2-fluoro-modified pyrimidines
gggagcgatcggctgtctgttcgtccccagactcgcccga

SEQ ID NO: 80 - RNA, 41 nt, synthetic construct
  source 1..41: mol_type = other RNA; note = Apt80 sequence
  modified_base 1..41: mod_base = OTHER; note = All pyrimidines are 2-fluoro-modified pyrimidines
gggagcgacggctgttctgttcgtccccagaactcgcccga

SEQ ID NO: 81 - RNA, 38 nt, synthetic construct
  source 1..38: mol_type = other RNA; note = Apt81 sequence
  modified_base 1..38: mod_base = OTHER; note = All pyrimidines are 2-fluoro-modified pyrimidines
ggaggacggtcctgtctgttcgtccccagactcgccga

SEQ ID NO: 82 - RNA, 38 nt, synthetic construct
  source 1..38: mol_type = other RNA; note = Apt82 sequence
  modified_base 1..32: mod_base = OTHER; note = All pyrimidines are 2-fluoro-modified pyrimidines
gaggacggtcctgttctgttcgtccccagaactcgcga

SEQ ID NO: 83 - RNA, 36 nt, synthetic construct
  source 1..36: mol_type = other RNA; note = Apt83 sequence
  modified_base 1..36: mod_base = OTHER; note = All pyrimidines are 2-fluoro-modified pyrimidines
gaggacggtcctgtctgttcgtccccagactcgcga

SEQ ID NO: 84 - RNA, 38 nt, synthetic construct
  source 1..38: mol_type = other RNA; note = Apt84 sequence
  modified_base 1..38: mod_base = OTHER; note = All pyrimidines are 2-fluoro-modified pyrimidines
gggagcggctgttctgttcgtccccagaactcgcccga

SEQ ID NO: 85 - RNA, 36 nt, synthetic construct
  source 1..36: mol_type = other RNA; note = Apt85 sequence
  modified_base 1..36: mod_base = OTHER; note = All pyrimidines are 2-fluoro-modified pyrimidines
gggagcggctgtctgttcgtccccagactcgcccga

SEQ ID NO: 86 - RNA, 40 nt, synthetic construct
  source 1..40: mol_type = other RNA; note = Apt86 sequence
  modified_base 1..40: mod_base = OTHER; note = All pyrimidines are 2-fluoro-modified pyrimidines
ggagcgatcggctgttctgttcgtccccagaactcgccga

SEQ ID NO: 87 - RNA, 38 nt, synthetic construct
  source 1..38: mol_type = other RNA; note = Apt87 sequence
  modified_base 1..38: mod_base = OTHER; note = All pyrimidines are 2-fluoro-modified pyrimidines
ggagcgatcggctgtctgttcgtccccagactcgccga

SEQ ID NO: 88 - RNA, 38 nt, synthetic construct
  source 1..38: mol_type = other RNA; note = Apt88 sequence
  modified_base 1..38: mod_base = OTHER; note = All pyrimidines are 2-fluoro-modified pyrimidines
gagcgatcggctgttctgttcgtccccagaactcgcga

SEQ ID NO: 89 - RNA, 36 nt, synthetic construct
  source 1..36: mol_type = other RNA; note = Apt89 sequence
  modified_base 1..36: mod_base = OTHER; note = All pyrimidines are 2-fluoro-modified pyrimidines
gagcgatcggctgtctgttcgtccccagactcgcga

SEQ ID NO: 90 - RNA, 39 nt, synthetic construct
  source 1..39: mol_type = other RNA; note = Apt90 sequence
  modified_base 1..39: mod_base = OTHER; note = All pyrimidines are 2-fluoro-modified pyrimidines
ggagcgacggctgttctgttcgtccccagaactcgccga

SEQ ID NO: 91 - RNA, 37 nt, synthetic construct
  source 1..37: mol_type = other RNA; note = Apt91 sequence
  modified_base 1..37: mod_base = OTHER; note = All pyrimidines are 2-fluoro-modified pyrimidines
gagcgacggctgttctgttcgtccccagaactcgcga

SEQ ID NO: 92 - RNA, 36 nt, synthetic construct
  source 1..36: mol_type = other RNA; note = Apt92 sequence
  modified_base 1..36: mod_base = OTHER; note = All pyrimidines are 2-fluoro-modified pyrimidines
ggagcggctgttctgttcgtccccagaactcgccga

SEQ ID NO: 93 - RNA, 34 nt, synthetic construct
  source 1..34: mol_type = other RNA; note = Apt93 sequence
  modified_base 1..34: mod_base = OTHER; note = All pyrimidines are 2-fluoro-modified pyrimidines
ggagcggctgtctgttcgtccccagactcgccga

SEQ ID NO: 94 - RNA, 34 nt, synthetic construct
  source 1..34: mol_type = other RNA; note = Apt94 sequence
  modified_base 1..34: mod_base = OTHER; note = All pyrimidines are 2-fluoro-modified pyrimidines
gagcggctgttctgttcgtccccagaactcgcga

SEQ ID NO: 95 - RNA, 32 nt, synthetic construct
  source 1..32: mol_type = other RNA; note = Apt95 sequence
  modified_base 1..32: mod_base = OTHER; note = All pyrimidines are 2-fluoro-modified pyrimidines
gagcggctgtctgttcgtccccagactcgcga

SEQ ID NO: 96 - RNA, 41 nt, synthetic construct
  source 1..41: mol_type = other RNA; note = Apt96 sequence
  modified_base 1..41: mod_base = OTHER; note = All pyrimidines are 2-fluoro-modified pyrimidines
gagcgacggctgtcgtctgttcgtccccagacgactcgcga

SEQ ID NO: 97 - RNA, 40 nt, synthetic construct
  source 1..40: mol_type = other RNA; note = Apt97 sequence
  modified_base 1..40: mod_base = OTHER; note = All pyrimidines are 2-fluoro-modified pyrimidines
ggagcggctgtcgtctgttcgtccccagacgactcgccga

SEQ ID NO: 98 - RNA, 38 nt, synthetic construct
  source 1..38: mol_type = other RNA; note = Apt98 sequence
  modified_base 1..38: mod_base = OTHER; note = All pyrimidines are 2-fluoro-modified pyrimidines
gagcggctgtcgtctgttcgtccccagacgactcgcga

SEQ ID NO: 99 - RNA, 42 nt, synthetic construct
  source 1..42: mol_type = other RNA; note = Apt99 sequence
  modified_base 1..42: mod_base = OTHER; note = All pyrimidines are 2-fluoro-modified pyrimidines
ggaggacgagcggtcctgtctgttcgtccccagactcgccga

SEQ ID NO: 100 - RNA, 42 nt, synthetic construct
  source 1..42: mol_type = other RNA; note = Apt100 sequence
  modified_base 1..42: mod_base = OTHER; note = All pyrimidines are 2-fluoro-modified pyrimidines
gaggacgagcggtcctgttctgttcgtccccagaactcgcga

SEQ ID NO: 101 - RNA, 40 nt, synthetic construct
  source 1..40: mol_type = other RNA; note = Apt101 sequence
  modified_base 1..40: mod_base = OTHER; note = All pyrimidines are 2-fluoro-modified pyrimidines
gaggacgagcggtcctgtctgttcgtccccagactcgcga

SEQ ID NO: 102 - RNA, 42 nt, synthetic construct
  source 1..42: mol_type = other RNA; note = Apt102 sequence
  modified_base 1..42: mod_base = OTHER; note = All pyrimidines are 2-fluoro-modified pyrimidines
gggagcgagcggctgttctgttcgtccccagaactcgcccga

SEQ ID NO: 103 - RNA, 40 nt, synthetic construct
  source 1..40: mol_type = other RNA; note = Apt103 sequence
  modified_base 1..40: mod_base = OTHER; note = All pyrimidines are 2-fluoro-modified pyrimidines
gggagcgagcggctgtctgttcgtccccagactcgcccga

SEQ ID NO: 104 - RNA, 40 nt, synthetic construct
  source 1..40: mol_type = other RNA; note = Apt104 sequence
  modified_base 1..40: mod_base = OTHER; note = All pyrimidines are 2-fluoro-modified pyrimidines
ggagcgagcggctgttctgttcgtccccagaactcgccga

SEQ ID NO: 105 - RNA, 38 nt, synthetic construct
  source 1..38: mol_type = other RNA; note = Apt105 sequence
  modified_base 1..38: mod_base = OTHER; note = All pyrimidines are 2-fluoro-modified pyrimidines
ggagcgagcggctgtctgttcgtccccagactcgccga

SEQ ID NO: 106 - RNA, 38 nt, synthetic construct
  source 1..38: mol_type = other RNA; note = Apt106 sequence
  modified_base 1..38: mod_base = OTHER; note = All pyrimidines are 2-fluoro-modified pyrimidines
gagcgagcggctgttctgttcgtccccagaactcgcga

SEQ ID NO: 107 - RNA, 36 nt, synthetic construct
  source 1..36: mol_type = other RNA; note = Apt107 sequence
  modified_base 1..36: mod_base = OTHER; note = All pyrimidines are 2-fluoro-modified pyrimidines
gagcgagcggctgtctgttcgtccccagactcgcga

SEQ ID NO: 108 - RNA, 42 nt, synthetic construct
  source 1..42: mol_type = other RNA; note = Apt108 sequence
  modified_base 1..42: mod_base = OTHER; note = All pyrimidines are 2-fluoro-modified pyrimidines
gagcgagcggctgtcgtctgttcgtccccagacgactcgcga

SEQ ID NO: 109 - RNA, 51 nt, synthetic construct
  source 1..51: mol_type = other RNA; note = AptP sequence
  modified_base 1..51: mod_base = OTHER; note = All pyrimidines are 2-fluoro-modified pyrimidines
gggaggacgatgcggtccttgtcgtcttgcgtccccagacgactcgcccga

SEQ ID NO: 110 - RNA, 25 nt, synthetic construct
  source 1..25: mol_type = other RNA; note = AptP (core) sequence
  modified_base 1..25: mod_base = OTHER; note = All pyrimidines are 2-fluoro-modified pyrimidines
gtcgtcttgcgtccccagacgactc

SEQ ID NO: 111 - RNA, 51 nt, synthetic construct
  source 1..51: mol_type = other RNA; note = Scramble sequence
  modified_base 1..51: mod_base = OTHER; note = All pyrimidines are 2-fluoro-modified pyrimidines
gcactcgctctcgggcttgggctctgcctgcacggtggacaacggctagca

SEQ ID NO: 112 - RNA, 44 nt, synthetic construct
  source 1..44: mol_type = other RNA; note = Apt49_UG sequence
  modified_base 1..44: mod_base = OTHER; note = All pyrimidines are 2-fluoro-modified pyrimidines
gggaggacgatcggtcctgtctgtgcgtccccagactcgcccga

SEQ ID NO: 113 - RNA, 44 nt, synthetic construct
  source 1..44: mol_type = other RNA; note = Apt49_GU sequence
  modified_base 1..44: mod_base = OTHER; note = All pyrimidines are 2-fluoro-modified pyrimidines
gggaggacgatcggtcctttctgttcgtccccagactcgcccga

SEQ ID NO: 114 - RNA, 44 nt, synthetic construct; identical to SEQ ID NO: 49
  source 1..44: mol_type = other RNA; note = PTO_Ends sequence
  misc_difference 1..44: note = G at position 1 and G at position 2 are linked through a phosphorothioate bond
  misc_difference 1..44: note = G at position 2 and G at position 3 are linked through a phosphorothioate bond
  misc_difference 1..44: note = G at position 42 and G at position 43 are linked through a phosphorothioate bond
  misc_difference 1..44: note = G at position 43 and A at position 44 are linked through a phosphorothioate bond

SEQ ID NO: 115 - RNA, 44 nt, synthetic construct; identical to SEQ ID NO: 49
  source 1..44: mol_type = other RNA; note = PTO_L1 sequence
  misc_difference 1..44: note = C at position 8 and G at position 9 are linked through a phosphorothioate bond
  misc_difference 1..44: note = G at position 9 and A at position 10 are linked through a phosphorothioate bond
  misc_difference 1..44: note = A at position 10 and T at position 11 are linked through a phosphorothioate bond
  misc_difference 1..44: note = T at position 11 and C at position 12 are linked through a phosphorothioate bond
  misc_difference 1..44: note = C at position 12 and G at position 13 are linked through a phosphorothioate bond
  misc_difference 1..44: note = G at position 13 and G at position 14 are linked through a phosphorothioate bond

SEQ ID NO: 116 - RNA, 44 nt, synthetic construct; identical to SEQ ID NO: 49
  source 1..44: mol_type = other RNA; note = PTO_L2 sequence
  misc_difference 1..44: note = G at position 23 and T at position 24 are linked through a phosphorothioate bond
  misc_difference 1..44: note = T at position 24 and T at position 25 are linked through a phosphorothioate bond
  misc_difference 1..44: note = T at position 25 and C at position 26 are linked through a phosphorothioate bond
  misc_difference 1..44: note = C at position 26 and G at position 27 are linked through a phosphorothioate bond
  misc_difference 1..44: note = G at position 27 and T at position 28 are linked through a phosphorothioate bond
  misc_difference 1..44: note = T at position 28 and C at position 29 are linked through a phosphorothioate bond
  misc_difference 1..44: note = C at position 29 and C at position 30 are linked through a phosphorothioate bond
  misc_difference 1..44: note = C at position 30 and C at position 31 are linked through a phosphorothioate bond
  misc_difference 1..44: note = C at position 31 and C at position 32 are linked through a phosphorothioate bond

SEQ ID NO: 117 - RNA, 44 nt, synthetic construct; identical to SEQ ID NO: 49
  source 1..44: mol_type = other RNA; note = PTO_L3 sequence
  misc_difference 1..44: note = C at position 36 and T at position 37 are linked through a phosphorothioate bond
  misc_difference 1..44: note = T at position 37 and C at position 38 are linked through a phosphorothioate bond
  misc_difference 1..44: note = C at position 38 and G at position 39 are linked through a phosphorothioate bond
  misc_difference 1..44: note = G at position 39 and C at position 40 are linked through a phosphorothioate bond

SEQ ID NO: 118 - RNA, 44 nt, synthetic construct; identical to SEQ ID NO: 49
  source 1..44: mol_type = other RNA; note = OMe_L1 sequence
  modified_base 1..44: mod_base = OTHER; note = G at position 9 is 2-O-methylated
  modified_base 1..44: mod_base = OTHER; note = A at position 10 is 2-O-methylated
  modified_base 1..44: mod_base = OTHER; note = T at position 11 is 2-O-methylated
  modified_base 1..44: mod_base = OTHER; note = C at position 12 is 2-O-methylated
  modified_base 1..44: mod_base = OTHER; note = G at position 13 is 2-O-methylated

SEQ ID NO: 119 - RNA, 44 nt, synthetic construct; identical to SEQ ID NO: 49
  source 1..44: mol_type = other RNA; note = OMe_L2.1 sequence
  modified_base 1..44: mod_base = OTHER; note = T at position 24 is 2-O-methylated
  modified_base 1..44: mod_base = OTHER; note = T at position 25 is 2-O-methylated
  modified_base 1..44: mod_base = OTHER; note = C at position 26 is 2-O-methylated
  modified_base 1..44: mod_base = OTHER; note = G at position 27 is 2-O-methylated

SEQ ID NO: 120 - RNA, 44 nt, synthetic construct; identical to SEQ ID NO: 49
  source 1..44: mol_type = other RNA; note = OMe_L2.2 sequence
  modified_base 1..44: mod_base = OTHER; note = T at position 28 is 2-O-methylated
  modified_base 1..44: mod_base = OTHER; note = C at position 29 is 2-O-methylated
  modified_base 1..44: mod_base = OTHER; note = C at position 30 is 2-O-methylated
  modified_base 1..44: mod_base = OTHER; note = C at position 31 is 2-O-methylated

SEQ ID NO: 121 - RNA, 44 nt, synthetic construct; identical to SEQ ID NO: 49
  source 1..44: mol_type = other RNA; note = OMe_L3 sequence
  modified_base 1..44: mod_base = OTHER; note = T at position 37 is 2-O-methylated
  modified_base 1..44: mod_base = OTHER; note = C at position 38 is 2-O-methylated
  modified_base 1..44: mod_base = OTHER; note = G at position 39 is 2-O-methylated

SEQ ID NO: 122 - RNA, 44 nt, synthetic construct; identical to SEQ ID NO: 49
  source 1..44: mol_type = other RNA; note = OMe_S1 sequence
  modified_base 1..44: mod_base = OTHER; note = G at position 1 is 2-O-methylated
  modified_base 1..44: mod_base = OTHER; note = G at position 2 is 2-O-methylated
  modified_base 1..44: mod_base = OTHER; note = G at position 3 is 2-O-methylated
  modified_base 1..44: mod_base = OTHER; note = C at position 40 is 2-O-methylated
  modified_base 1..44: mod_base = OTHER; note = C at position 41 is 2-O-methylated
  modified_base 1..44: mod_base = OTHER; note = C at position 42 is 2-O-methylated

SEQ ID NO: 123 - RNA, 44 nt, synthetic construct; identical to SEQ ID NO: 49
  source 1..44: mol_type = other RNA; note = OMe_S2 sequence
  modified_base 1..44: mod_base = OTHER; note = A at position 4 is 2-O-methylated
  modified_base 1..44: mod_base = OTHER; note = G at position 5 is 2-O-methylated
  modified_base 1..44: mod_base = OTHER; note = G at position 6 is 2-O-methylated
  modified_base 1..44: mod_base = OTHER; note = A at position 7 is 2-O-methylated
  modified_base 1..44: mod_base = OTHER; note = C at position 8 is 2-O-methylated
  modified_base 1..44: mod_base = OTHER; note = G at position 14 is 2-O-methylated
  modified_base 1..44: mod_base = OTHER; note = T at position 15 is 2-O-methylated
  modified_base 1..44: mod_base = OTHER; note = C at position 16 is 2-O-methylated
  modified_base 1..44: mod_base = OTHER; note = C at position 17 is 2-O-methylated
  modified_base 1..44: mod_base = OTHER; note = T at position 18 is 2-O-methylated

SEQ ID NO: 124 - RNA, 44 nt, synthetic construct; identical to SEQ ID NO: 49
  source 1..44: mol_type = other RNA; note = OMe_S3 sequence
  modified_base 1..44: mod_base = OTHER; note = G at position 19 is 2-O-methylated
  modified_base 1..44: mod_base = OTHER; note = T at position 20 is 2-O-methylated
  modified_base 1..44: mod_base = OTHER; note = C at position 21 is 2-O-methylated
  modified_base 1..44: mod_base = OTHER; note = T at position 22 is 2-O-methylated
  modified_base 1..44: mod_base = OTHER; note = G at position 23 is 2-O-methylated
  modified_base 1..44: mod_base = OTHER; note = C at position 32 is 2-O-methylated
  modified_base 1..44: mod_base = OTHER; note = A at position 33 is 2-O-methylated
  modified_base 1..44: mod_base = OTHER; note = G at position 34 is 2-O-methylated
  modified_base 1..44: mod_base = OTHER; note = A at position 35 is 2-O-methylated

SEQ ID NO: 125 - RNA, 44 nt, synthetic construct; identical to SEQ ID NO: 49
  source 1..44: mol_type = other RNA; note = OMe_1 sequence
  modified_base 1..44: mod_base = OTHER; note = C at position 8 is 2-O-methylated

SEQ ID NO: 126 - RNA, 44 nt, synthetic construct; identical to SEQ ID NO: 49
  source 1..44: mol_type = other RNA; note = OMe_2 sequence
  modified_base 1..44: mod_base = OTHER; note = T at position 11 is 2-O-methylated

SEQ ID NO: 127 - RNA, 44 nt, synthetic construct; identical to SEQ ID NO: 49
  source 1..44: mol_type = other RNA; note = OMe_3 sequence
  modified_base 1..44: mod_base = OTHER; note = C at position 12 is 2-O-methylated

SEQ ID NO: 128 - RNA, 44 nt, synthetic construct; identical to SEQ ID NO: 49
  source 1..44: mol_type = other RNA; note = OMe_4 sequence
  modified_base 1..44: mod_base = OTHER; note = T at position 15 is 2-O-methylated

SEQ ID NO: 129 - RNA, 44 nt, synthetic construct; identical to SEQ ID NO: 49
  source 1..44: mol_type = other RNA; note = OMe_5 sequence
  modified_base 1..44: mod_base = OTHER; note = C at position 16 is 2-O-methylated

SEQ ID NO: 130 - RNA, 44 nt, synthetic construct; identical to SEQ ID NO: 49
  source 1..44: mol_type = other RNA; note = OMe_6 sequence
  modified_base 1..44: mod_base = OTHER; note = C at position 17 is 2-O-methylated

SEQ ID NO: 131 - RNA, 44 nt, synthetic construct; identical to SEQ ID NO: 49
  source 1..44: mol_type = other RNA; note = OMe_7 sequence
  modified_base 1..44: mod_base = OTHER; note = T at position 18 is 2-O-methylated

SEQ ID NO: 132 - RNA, 44 nt, synthetic construct; identical to SEQ ID NO: 49
  source 1..44: mol_type = other RNA; note = OMe_8 sequence
  modified_base 1..44: mod_base = OTHER; note = T at position 20 is 2-O-methylated

SEQ ID NO: 133 - RNA, 44 nt, synthetic construct; identical to SEQ ID NO: 49
  source 1..44: mol_type = other RNA; note = OMe_9 sequence
  modified_base 1..44: mod_base = OTHER; note = C at position 21 is 2-O-methylated

SEQ ID NO: 134 - RNA, 44 nt, synthetic construct; identical to SEQ ID NO: 49
  source 1..44: mol_type = other RNA; note = OMe_10 sequence
  modified_base 1..44: mod_base = OTHER; note = T at position 22 is 2-O-methylated

SEQ ID NO: 135 - RNA, 44 nt, synthetic construct; identical to SEQ ID NO: 49
  source 1..44: mol_type = other RNA; note = OMe_11 sequence
  modified_base 1..44: mod_base = OTHER; note = T at position 24 is 2-O-methylated

SEQ ID NO: 136 - RNA, 44 nt, synthetic construct; identical to SEQ ID NO: 49
  source 1..44: mol_type = other RNA; note = OMe_12 sequence
  modified_base 1..44: mod_base = OTHER; note = T at position 25 is 2-O-methylated

SEQ ID NO: 137 - RNA, 44 nt, synthetic construct; identical to SEQ ID NO: 49
  source 1..44: mol_type = other RNA; note = OMe_13 sequence
  modified_base 1..44: mod_base = OTHER; note = C at position 26 is 2-O-methylated

SEQ ID NO: 138 - RNA, 44 nt, synthetic construct; identical to SEQ ID NO: 49
  source 1..44: mol_type = other RNA; note = OMe_14 sequence
  modified_base 1..44: mod_base = OTHER; note = T at position 28 is 2-O-methylated

SEQ ID NO: 139 - RNA, 44 nt, synthetic construct; identical to SEQ ID NO: 49
  source 1..44: mol_type = other RNA; note = OMe_15 sequence
  modified_base 1..44: mod_base = OTHER; note = C at position 29 is 2-O-methylated

SEQ ID NO: 140 - RNA, 44 nt, synthetic construct; identical to SEQ ID NO: 49
  source 1..44: mol_type = other RNA; note = OMe_16 sequence
  modified_base 1..44: mod_base = OTHER; note = C at position 30 is 2-O-methylated

SEQ ID NO: 141 - RNA, 44 nt, synthetic construct; identical to SEQ ID NO: 49
  source 1..44: mol_type = other RNA; note = OMe_17 sequence
  modified_base 1..44: mod_base = OTHER; note = C at position 31 is 2-O-methylated

SEQ ID NO: 142 - RNA, 44 nt, synthetic construct; identical to SEQ ID NO: 49
  source 1..44: mol_type = other RNA; note = OMe_18 sequence
  modified_base 1..44: mod_base = OTHER; note = C at position 32 is 2-O-methylated

SEQ ID NO: 143 - RNA, 44 nt, synthetic construct; identical to SEQ ID NO: 49
  source 1..44: mol_type = other RNA; note = OMe_19 sequence
  modified_base 1..44: mod_base = OTHER; note = C at position 36 is 2-O-methylated

SEQ ID NO: 144 - RNA, 44 nt, synthetic construct; identical to SEQ ID NO: 49
  source 1..44: mol_type = other RNA; note = OMe_20 sequence
  modified_base 1..44: mod_base = OTHER; note = T at position 37 is 2-O-methylated

SEQ ID NO: 145 - RNA, 44 nt, synthetic construct; identical to SEQ ID NO: 49
  source 1..44: mol_type = other RNA; note = OMe_21 sequence
  modified_base 1..44: mod_base = OTHER; note = C at position 38 is 2-O-methylated

SEQ ID NO: 146 - RNA, 44 nt, synthetic construct; identical to SEQ ID NO: 49
  source 1..44: mol_type = other RNA; note = OMe_22 sequence
  modified_base 1..44: mod_base = OTHER; note = C at position 40 is 2-O-methylated

SEQ ID NO: 147 - RNA, 44 nt, synthetic construct; identical to SEQ ID NO: 49
  source 1..44: mol_type = other RNA; note = OMe_23 sequence
  modified_base 1..44: mod_base = OTHER; note = C at position 41 is 2-O-methylated

SEQ ID NO: 148 - RNA, 44 nt, synthetic construct; identical to SEQ ID NO: 49
  source 1..44: mol_type = other RNA; note = OMe_24 sequence
  modified_base 1..44: mod_base = OTHER; note = C at position 42 is 2-O-methylated